European Patent Application EP 4 397 683 A1, published July 10, 2024. Title: ANTI-HUMAN INTERLEUKIN-33 MONOCLONAL ANTIBODY AND USE THEREOF. Applicant: Qyuns Therapeutics Co., Ltd. The sequence listing filed with the application follows.

SEQUENCE LISTING (11 sequences)

SEQ ID NO: 1 - protein, 5 aa, Artificial sequence
  synthetic
SYHMI

SEQ ID NO: 2 - protein, 16 aa, Artificial sequence
  synthetic
VIYPNSNIYYATWAKG

SEQ ID NO: 3 - protein, 12 aa, Artificial sequence
  synthetic
TIYVHVYSALSI

SEQ ID NO: 4 - protein, 11 aa, Artificial sequence
  synthetic
QASESVLNEVS

SEQ ID NO: 5 - protein, 7 aa, Artificial sequence
  synthetic
FASKLAS

SEQ ID NO: 6 - protein, 12 aa, Artificial sequence
  synthetic
QQDWSMDNIDNA

SEQ ID NO: 7 - protein, 120 aa, Artificial sequence
  synthetic
EVQLVESGGGLVQPGGSLRLSCAASGFSLSSYHMIWVRQAPGKGLEWVGVIYPNSNIYYATWAKGRFTISRDNSKNTLYLQMNSLRAEDTAVYYCARTIYVHVYSALSIWGQGTLVTVSS

SEQ ID NO: 8 - protein, 110 aa, Artificial sequence
  synthetic
AFQMTQSPSSVSASVGDRVTITCQASESVLNEVSWYQQKPGKAPKLLIYFASKLASGVPSRFSGSGSGTDFTLTISSLQPEDFATYYCQQDWSMDNIDNAFGGGTKVEIK

SEQ ID NO: 9 - protein, 159 aa, Artificial sequence
  synthetic
SITGISPITEYLASLSTYNDQSITFALEDESYEIYVEDLKKDEKKDKVLLSYYESQHPSNESGDGVDGKMLMVTLSPTKDFWLHANNKEHSVELHKCEKPLPDQAFFVLHNMHSNCVSFECKTDPGVFIGVKDNHLALIKVDSSENLCTENILFKLSET

SEQ ID NO: 10 - protein, 450 aa, Artificial sequence
  synthetic
EVQLVESGGGLVQPGGSLRLSCAASGFSLSSYHMIWVRQAPGKGLEWVGVIYPNSNIYYATWAKGRFTISRDNSKNTLYLQMNSLRAEDTAVYYCARTIYVHVYSALSIWGQGTLVTVSSASTKGPSVFPLAPSSKSTSGGTAALGCLVKDYFPEPVTVSWNSGALTSGVHTFPAVLQSSGLYSLSSVVTVPSSSLGTQTYICNVNHKPSNTKVDKKVEPKSCDKTHTCPPCPAPELLGGPSVFLFPPKPKDTLMISRTPEVTCVVVDVSHEDPEVKFNWYVDGVEVHNAKTKPREEQYNSTYRVVSVLTVLHQDWLNGKEYKCKVSNKALPAPIEKTISKAKGQPREPQVYTLPPSRDELTKNQVSLTCLVKGFYPSDIAVEWESNGQPENNYKTTPPVLDSDGSFFLYSKLTVDKSRWQQGNVFSCSVMHEALHNHYTQKSLSLSPGK

SEQ ID NO: 11 - protein, 217 aa, Artificial sequence
  synthetic
AFQMTQSPSSVSASVGDRVTITCQASESVLNEVSWYQQKPGKAPKLLIYFASKLASGVPSRFSGSGSGTDFTLTISSLQPEDFATYYCQQDWSMDNIDNAFGGGTKVEIKRTVAAPSVFIFPPSDEQLKSGTASVVCLLNNFYPREAKVQWKVDNALQSGNSQESVTEQDSKDSTYSLSSTLTLSKADYEKHKVYACEVTHQGLSSPVTKSFNRGEC